European Patent Specification EP 4 149 961 B1, published January 28, 2026. Title: JNK3 inhibitory peptides. Applicant: Università degli Studi di Milano Università degli Studi di Roma "Tor Vergata" Università Politecnica delle Marche. The sequence listing filed with the application follows.

SEQUENCE LISTING (5 sequences)

SEQ ID NO: 1 - protein, 56 aa, Artificial Sequence
  Designed peptide based on size and structure to act in the interaction among beta-arrestin-2 and JNK3
SDRSLHLEANEKGENVNVHVTKTRADKSKIKVSVRQYADINEKGEAQYKCPVAQLE

SEQ ID NO: 2 - protein, 50 aa, Artificial Sequence
  Designed peptide based on size and structure to act in the interaction among beta-arrestin-2 and JNK3
SDRSLHLEAEKGNVNVHVTKTEKGKIKVSVRQYADIEKGAQYKCPVAQLE

SEQ ID NO: 3 - protein, 50 aa, Artificial Sequence
  Designed peptide based on size and structure to act in the interaction among beta-arrestin-2 and JNK3
SDRSLHLEAEKGNVNVHVTKTADKKIKVSVRQYADIEKGAQYKCPVAQLE

SEQ ID NO: 4 - protein, 56 aa, Artificial Sequence
  Designed peptide based on size and structure to act in the interaction among beta-arrestin-2 and JNK3
SDRSLHLEANEKGENVNVHVTKTNEKGEKIKVSVRQYADINEKGEAQYKCPVAQLE

SEQ ID NO: 5 - protein, 11 aa, Artificial Sequence
  Protein TAT
YGRKKRRQRRR